European Patent Specification EP 3 702 360 B1, published September 9, 2026. Title: NOVEL PROCESSES FOR THE PRODUCTION OF OLIGONUCLEOTIDES. Applicant: GlaxoSmithKline Intellectual Property Development Limited. The sequence listing filed with the application follows.

SEQUENCE LISTING (62 sequences)

SEQ ID NO: 1 - DNA, 20 bp, Artificial sequence
  Example 1 desired product oligonucleotide sequence ("target")
ggccaaacctcggcttacct

SEQ ID NO: 2 - DNA, 23 bp, Artificial sequence
  Example 1-4, 6, 10 and 11 template oligonucleotide sequence
tttaggtaagccgaggtttggcc

SEQ ID NO: 3 - protein, 487 aa, Enterobacteria phage T4
MILKILNEIASIGSTKQKQAILEKNKDNELLKRVYRLTYSRGLQYYIKKWPKPGIATQSFGMLTLTDMLDFIEFTLATRKLTGNAAIEELTGYITDGKKDDVEVLRRVMMRDLECGASVSIANKVWPGLIPEQPQMLASSYDEKGINKNIKFPAFAQLKADGARCFAEVRGDELDDVRLLSRAGNEYLGLDLLKEELIKMTAEARQIHPEGVLIDGELVYHEQVKKEPEGLDFLFDAYPENSKAKEFAEVAESRTASNGIANKSLKGTISEKEAQCMKFQVWDYVPLVEIYSLPAFRLKYDVRFSKLEQMTSGYDKVILIENQVVNNLDEAKVIYKKYIDQGLEGIILKNIDGLWENARSKNLYKFKEVIDVDLKIVGIYPHRKDPTKAGGFILESECGKIKVNAGSGLKDKAGVKSHELDRTRIMENQNYYIGKILECECNGWLKSDGRTDYVKLFLPIAIRLREDKTKANTFEDVFGDFHEVTGL

SEQ ID NO: 4 - protein, 488 aa, Artificial sequence
  Wild type T4 DNA ligase protein sequence (when fused to CBD)
GSILKILNEIASIGSTKQKQAILEKNKDNELLKRVYRLTYSRGLQYYIKKWPKPGIATQSFGMLTLTDMLDFIEFTLATRKLTGNAAIEELTGYITDGKKDDVEVLRRVMMRDLECGASVSIANKVWPGLIPEQPQMLASSYDEKGINKNIKFPAFAQLKADGARCFAEVRGDELDDVRLLSRAGNEYLGLDLLKEELIKMTAEARQIHPEGVLIDGELVYHEQVKKEPEGLDFLFDAYPENSKAKEFAEVAESRTASNGIANKSLKGTISEKEAQCMKFQVWDYVPLVEIYSLPAFRLKYDVRFSKLEQMTSGYDKVILIENQVVNNLDEAKVIYKKYIDQGLEGIILKNIDGLWENARSKNLYKFKEVIDVDLKIVGIYPHRKDPTKAGGFILESECGKIKVNAGSGLKDKAGVKSHELDRTRIMENQNYYIGKILECECNGWLKSDGRTDYVKLFLPIAIRLREDKTKANTFEDVFGDFHEVTGL

SEQ ID NO: 5 - RNA, 20 nt, Artificial sequence
  Example 2 target sequence
ggccaaaccucggcuuaccu

SEQ ID NO: 6 - protein, 482 aa, Enterobacteria phase CC31
MILDIINEIASIGSTKEKEAIIRRHKDNELLKRVFRMTYDGKLQYYIKKWDTRPKGDIHLTLEDMLYLLEEKLAKRVVTGNAAKEKLEIALSQTSDADAEVVKKVLLRDLRCGASRSIANKVWKNLIPEQPQMLASSYDEKGIEKNIKFPAFAQLKADGARAFAEVRGDELDDVKILSRAGNEYLGLDLLKQQLIEMTKEARERHPGGVMIDGELVYHASTLPAGPLDDIFGDLPELSKAKEFKEESRTMSNGLANKSLKGTISAKEAAGMKFQVWDYVPLDVVYSEGKQSGFAYDVRFRALELMVQGYSQMILIENHIVHNLDEAKVIYRKYVDEGLEGIILKNIGAFWENTRSKNLYKFKEVITIDLRIVDIYEHSKQPGKAGGFYLESECGLIKVKAGSGLKDKPGKDAHELDRTRIWENKNDYIGGVLESECNGWLAAEGRTDYVKLFLPIAIKMRRDKDVANTFADIWGDFHEVTGL

SEQ ID NO: 7 - protein, 483 aa, Artificial sequence
  Wild-type Enterobacteria phage CC31 DNA ligase protein sequence (when fused to CBD)
GSILDIINEIASIGSTKEKEAIIRRHKDNELLKRVFRMTYDGKLQYYIKKWDTRPKGDIHLTLEDMLYLLEEKLAKRVVTGNAAKEKLEIALSQTSDADAEVVKKVLLRDLRCGASRSIANKVWKNLIPEQPQMLASSYDEKGIEKNIKFPAFAQLKADGARAFAEVRGDELDDVKILSRAGNEYLGLDLLKQQLIEMTKEARERHPGGVMIDGELVYHASTLPAGPLDDIFGDLPELSKAKEFKEESRTMSNGLANKSLKGTISAKEAAGMKFQVWDYVPLDVVYSEGKQSGFAYDVRFRALELMVQGYSQMILIENHIVHNLDEAKVIYRKYVDEGLEGIILKNIGAFWENTRSKNLYKFKEVITIDLRIVDIYEHSKQPGKAGGFYLESECGLIKVKAGSGLKDKPGKDAHELDRTRIWENKNDYIGGVLESECNGWLAAEGRTDYVKLFLPIAIKMRRDKDVANTFADIWGDFHEVTGL

SEQ ID NO: 8 - protein, 497 aa, Shigella phage Shf125875
MILDILNQIAAIGSTKTKQEILKKNKDNKLLERVYRLTYARGIQYYIKKWPGPGERSQAYGLLELDDMLDFIEFTLATRKLTGNAAIKELMGYIADGKPDDVEVLRRVMMRDLEVGASVSIANKVWPGLIQLQPQMLASAYDEKLITKNIKWPAFAQLKADGARCFAEVRDDGVQFFSRAGNEYHGLTLLADELMEMTKEARERHPNGVLIDGELVYHSFDIKKAVSSGNDLSFLFGDNEESEEVQVADRSTSNGLANKSLQGTISPKEAEGMVLQAWDYVPLDEVYSDGKIKGQKYDVRFAALENMAEGFKRIEPIENQLVHNLDEAKVVYKKYVDQGLEGIILKNRDSYWENKRSKNLIKFKEVIDIALEVVGYYEHSKDPNKLGGVELVSRCRRITTDCGSGFKDTTHKTVDGVKVLIPLDERHDLDRERLMAEAREGKLIGRIADCECNGWVHSKGREGTVGIFLPIIKGFRFDKTEADSFEDVFGPWSQTGL

SEQ ID NO: 9 - protein, 498 aa, Artificial sequence
  Wild-type Shigella phage Shf125875 DNA ligase protein sequence (when fused to CBD)
GSILDILNQIAAIGSTKTKQEILKKNKDNKLLERVYRLTYARGIQYYIKKWPGPGERSQAYGLLELDDMLDFIEFTLATRKLTGNAAIKELMGYIADGKPDDVEVLRRVMMRDLEVGASVSIANKVWPGLIQLQPQMLASAYDEKLITKNIKWPAFAQLKADGARCFAEVRDDGVQFFSRAGNEYHGLTLLADELMEMTKEARERHPNGVLIDGELVYHSFDIKKAVSSGNDLSFLFGDNEESEEVQVADRSTSNGLANKSLQGTISPKEAEGMVLQAWDYVPLDEVYSDGKIKGQKYDVRFAALENMAEGFKRIEPIENQLVHNLDEAKVVYKKYVDQGLEGIILKNRDSYWENKRSKNLIKFKEVIDIALEVVGYYEHSKDPNKLGGVELVSRCRRITTDCGSGFKDTTHKTVDGVKVLIPLDERHDLDRERLMAEAREGKLIGRIADCECNGWVHSKGREGTVGIFLPIIKGFRFDKTEADSFEDVFGPWSQTGL

SEQ ID NO: 10 - protein, 487 aa, Artificial sequence
  Mutant ligase (T4 backbone) protein sequence
MILKILNEIASIGSTKQKQAILEKNKDNELLKRVYRLTYSRGLQYYIKKWPKPGIATQSFGMLTLTDMLDFIEFTLATRKLTGNAAIEELTGYITDGKKDDVEVLRRVMMRDLECGASVSIANKVWPGLIPEQPQMLASSYDEKGINKNIKFPAFAQLKADGARCFAEVRGDELDDVRLLSRAGNEYLGLDLLKEELIKMTAEARQIHPEGVLIDGELVYHEQVKKEPEGLDFLFDAYPENSKAKEFAEVAESRTASNGIANKSLKGTISEKEAQCMKFQVWDYVPLVEIYSLPAFRLKYDVRFSKLEQMTSGYDKVILIENQVVNNLDEAKVIYKKYIDQGLEGIILKNIDGLWENARSKNLYKFKRVIDVDLKIVGIYPHRKDPTKAGGFILESECGKIKVNAGSGLKDKAGVKSHELDRTRIMENQNYYIGKILECECNGWLKSDGRTDYVKLFLPIAIRLREDKTKANTFEDVFGDFHEVTGL

SEQ ID NO: 11 - protein, 487 aa, Artificial sequence
  Mutant ligase (T4 backbone) protein sequence
MILKILNEIASIGSTKQKQAILEKNKDNELLKRVYRLTYSRGLQYYIKKWPKPGIATQSFGMLTLTDMLDFIEFTLATRKLTGNAAIEELTGYITDGKKDDVEVLRRVMMRDLECGASVSIANKVWPGLIPEQPQMLASSYDEKGINKNIKFPAFAQLKADGARCFAEVRGDELDDVRLLSRAGNEYLGLDLLKEELIKMTAEARQIHPEGVLIDGELVYHEQVKKEPEGLDFLFDAYPENSKAKEFAEVAESRTASNGIANKSLKGTISEKEAQCMKFQVWDYVPLVEIYSLPAFRLKYDVRFSKLEQMTSGYDKVILIENQVVNNLDEAKVIYKKYIDQGLEGIILKNIDGLWENARSKNLYKFKGVIDVDLKIVGIYPHRKDPTKAGGFILESECGKIKVNAGSGLKDKAGVKSHELDRTRIMENQNYYIGKILECECNGWLKSDGRTDYVKLFLPIAIRLREDKTKANTFEDVFGDFHEVTGL

SEQ ID NO: 12 - protein, 487 aa, Artificial sequence
  Mutant ligase (T4 backbone) protein sequence
MILKILNEIASIGSTKQKQAILEKNKDNELLKRVYRLTYSRGLQYYIKKWPKPGIATQSFGMLTLTDMLDFIEFTLATRKLTGNAAIEELTGYITDGKKDDVEVLRRVMMRDLECGASVSIANKVWPGLIPEQPQMLASSYDEKGINKNIKFPAFAQLKADGARCFAEVRGDELDDVRLLSRAGNEYLGLDLLKEELIKMTAEARQIHPEGVLIDGELVYHEQVKKEPEGLDFLFDAYPENSKAKEFAEVAESRTASNGIANKSLKGTISEKEAQCMKFQVWDYVPLVEIYSLPAFRLKYDVRFSKLEQMTSGYDKVILIENQVVNNLDEAKVIYKKYIDQGLEGIILKNIDGLWENARSKNLYKFKKVIDVDLKIVGIYPHRKDPTKAGGFILESECGKIKVNAGSGLKDKAGVKSHELDRTRIMENQNYYIGKILECECNGWLKSDGRTDYVKLFLPIAIRLREDKTKANTFEDVFGDFHEVTGL

SEQ ID NO: 13 - protein, 487 aa, Artificial sequence
  Mutant ligase (T4 backbone) protein sequence
MILKILNEIASIGSTKQKQAILEKNKDNELLKRVYRLTYSRGLQYYIKKWPKPGIATQSFGMLTLTDMLDFIEFTLATRKLTGNAAIEELTGYITDGKKDDVEVLRRVMMRDLECGASVSIANKVWPGLIPEQPQMLASSYDEKGINKNIKFPAFAQLKADGARCFAEVRGDELDDVRLLSRAGNEYLGLDLLKEELIKMTAEARQIHPEGVLIDGELVYHEQVKKEPEGLDFLFDAYPENSKAKEFAEVAESRTASNGIANKSLKGTISEKEAQCMKFQVWDYVPLVEIYSLPAFRLKYDVRFSKLEQMTSGYDKVILIENQVVNNLDEAKVIYKKYIDQGLEGIILKNIDGLWENARSKNLYKFKEVILVDLKIVGIYPHRKDPTKAGGFILESECGKIKVNAGSGLKDKAGVKSHELDRTRIMENQNYYIGKILECECNGWLKSDGRTDYVKLFLPIAIRLREDKTKANTFEDVFGDFHEVTGL

SEQ ID NO: 14 - protein, 487 aa, Artificial sequence
  Mutant ligase (T4 backbone) protein sequence
MILKILNEIASIGSTKQKQAILEKNKDNELLKRVYRLTYSRGLQYYIKKWPKPGIATQSFGMLTLTDMLDFIEFTLATRKLTGNAAIEELTGYITDGKKDDVEVLRRVMMRDLECGASVSIANKVWPGLIPEQPQMLASSYDEKGINKNIKFPAFAQLKADGARCFAEVRGDELDDVRLLSRAGNEYLGLDLLKEELIKMTAEARQIHPEGVLIDGELVYHEQVKKEPEGLDFLFDAYPENSKAKEFAEVAESRTASNGIANKSLKGTISEKEAQCMKFQVWDYVPLVEIYSLPAFRLKYDVRFSKLEQMTSGYDKVILIENQVVNNLDEAKVIYKKYIDQGLEGIILKNIDGLWENARSKNLYKFKEVIQVDLKIVGIYPHRKDPTKAGGFILESECGKIKVNAGSGLKDKAGVKSHELDRTRIMENQNYYIGKILECECNGWLKSDGRTDYVKLFLPIAIRLREDKTKANTFEDVFGDFHEVTGL

SEQ ID NO: 15 - protein, 487 aa, Artificial sequence; identical to SEQ ID NO: 14
  Mutant ligase (T4 backbone) protein sequence

SEQ ID NO: 16 - protein, 487 aa, Artificial sequence
  Mutant ligase (T4 backbone) protein sequence
MILKILNEIASIGSTKQKQAILEKNKDNELLKRVYRLTYSRGLQYYIKKWPKPGIATQSFGMLTLTDMLDFIEFTLATRKLTGNAAIEELTGYITDGKKDDVEVLRRVMMRDLECGASVSIANKVWPGLIPEQPQMLASSYDEKGINKNIKFPAFAQLKADGARCFAEVRGDELDDVRLLSRAGNEYLGLDLLKEELIKMTAEARQIHPEGVLIDGELVYHEQVKKEPEGLDFLFDAYPENSKAKEFAEVAESRTASNGIANKSLKGTISEKEAQCMKFQVWDYVPLVEIYSLPAFRLKYDVRFSKLEQMTSGYDKVILIENQVVNNLDEAKVIYKKYIDQGLEGIILKNIDGLWENARSKNLYKFKEVIVVDLKIVGIYPHRKDPTKAGGFILESECGKIKVNAGSGLKDKAGVKSHELDRTRIMENQNYYIGKILECECNGWLKSDGRTDYVKLFLPIAIRLREDKTKANTFEDVFGDFHEVTGL

SEQ ID NO: 17 - protein, 487 aa, Artificial sequence
  Mutant ligase (T4 backbone) protein sequence
MILKILNEIASIGSTKQKQAILEKNKDNELLKRVYRLTYSRGLQYYIKKWPKPGIATQSFGMLTLTDMLDFIEFTLATRKLTGNAAIEELTGYITDGKKDDVEVLRRVMMRDLECGASVSIANKVWPGLIPEQPQMLASSYDEKGINKNIKFPAFAQLKADGARCFAEVRGDELDDVRLLSRAGNEYLGLDLLKEELIKMTAEARQIHPEGVLIDGELVYHEQVKKEPEGLDFLFDAYPENSKAKEFAEVAESRTASNGIANKSLKGTISEKEAQCMKFQVWDYVPLVEIYSLPAFRLKYDVRFSKLEQMTSGYDKVILIENQVVNNLDEAKVIYKKYIDQGLEGIILKNIDGLWENARSKNLYKFKEVIRVDLKIVGIYPHRKDPTKAGGFILESECGKIKVNAGSGLKDKAGVKSHELDRTRIMENQNYYIGKILECECNGWLKSDGRTDYVKLFLPIAIRLREDKTKANTFEDVFGDFHEVTGL

SEQ ID NO: 18 - protein, 487 aa, Artificial sequence
  Mutant ligase (T4 backbone) protein sequence
MILKILNEIASIGSTKQKQAILEKNKDNELLKRVYRLTYSRGLQYYIKKWPKPGIATQSFGMLTLTDMLDFIEFTLATRKLTGNAAIEELTGYITDGKKDDVEVLRRVMMRDLECGASVSIANKVWPGLIPEQPQMLASSYDEKGINKNIKFPAFAQLKADGARCFAEVRGDELDDVRLLSRAGNEYLGLDLLKEELIKMTAEARQIHPEGVLIDGELVYHEQVKKEPEGLDFLFDAYPENSKAKEFAEVAESRTASNGIANKSLKGTISEKEAQCMKFQVWDYVPLVEIYSLPAFRLKYDVRFSKLEQMTSGYDKVILIENQVVNNLDEAKVIYKKYIDQGLEGIILKNIDGLWENARSKNLYKFKEAIDVDLKIVGIYPHRKDPTKAGGFILESECGKIKVNAGSGLKDKAGVKSHELDRTRIMENQNYYIGKILECECNGWLKSDGRTDYVKLFLPIAIRLREDKTKANTFEDVFGDFHEVTGL

SEQ ID NO: 19 - protein, 487 aa, Artificial sequence
  Mutant ligase (T4 backbone) protein sequence
MILKILNEIASIGSTKQKQAILEKNKDNELLKRVYRLTYSRGLQYYIKKWPKPGIATQSFGMLTLTDMLDFIEFTLATRKLTGNAAIEELTGYITDGKKDDVEVLRRVMMRDLECGASVSIANKVWPGLIPEQPQMLASSYDEKGINKNIKFPAFAQLKADGARCFAEVRGDELDDVRLLSRAGNEYLGLDLLKEELIKMTAEARQIHPEGVLIDGELVYHEQVKKEPEGLDFLFDAYPENSKAKEFAEVAESRTASNGIANKSLKGTISEKEAQCMKFQVWDYVPLVEIYSLPAFRLKYDVRFSKLEQMTSGYDKVILIENQVVNNLDEAKVIYKKYIDQGLEGIILKNIDGLWENARSKNLYKFKEKIDVDLKIVGIYPHRKDPTKAGGFILESECGKIKVNAGSGLKDKAGVKSHELDRTRIMENQNYYIGKILECECNGWLKSDGRTDYVKLFLPIAIRLREDKTKANTFEDVFGDFHEVTGL

SEQ ID NO: 20 - protein, 487 aa, Artificial sequence
  Mutant ligase (T4 backbone) protein sequence
MILKILNEIASIGSTKQKQAILEKNKDNELLKRVYRLTYSRGLQYYIKKWPKPGIATQSFGMLTLTDMLDFIEFTLATRKLTGNAAIEELTGYITDGKKDDVEVLRRVMMRDLECGASVSIANKVWPGLIPEQPQMLASSYDEKGINKNIKFPAFAQLKADGARCFAEVRGDELDDVRLLSRAGNEYLGLDLLKEELIKMTAEARQIHPEGVLIDGELVYHEQVKKEPEGLDFLFDAYPENSKAKEFAEVAESRTASNGIANKSLKGTISEKEAQCMKFQVWDYVPLVEIYSLPAFRLKYDVRFSKLEQMTSGYDKVILIENQVVNNLDEAKVIYKKYIDQGLEGIILKNIDGLWENARSKNLYKFKRVIVVDLKIVGIYPHRKDPTKAGGFILESECGKIKVNAGSGLKDKAGVKSHELDRTRIMENQNYYIGKILECECNGWLKSDGRTDYVKLFLPIAIRLREDKTKANTFEDVFGDFHEVTGL

SEQ ID NO: 21 - protein, 487 aa, Artificial sequence
  Mutant ligase (T4 backbone) protein sequence
MILKILNEIASIGSTKQKQAILEKNKDNELLKRVYRLTYSRGLQYYIKKWPKPGIATQSFGMLTLTDMLDFIEFTLATRKLTGNAAIEELTGYITDGKKDDVEVLRRVMMRDLECGASVSIANKVWPGLIPEQPQMLASSYDEKGINKNIKFPAFAQLKADGARCFAEVRGDELDDVRLLSRAGNEYLGLDLLKEELIKMTAEARQIHPEGVLIDGELVYHEQVKKEPEGLDFLFDAYPENSKAKEFAEVAESRTASNGIANKSLKGTISEKEAQCMKFQVWDYVPLVEIYSLPAFRLKYDVRFSKLEQMTSGYDKVILIENQVVNNLDEAKVIYKKYIDQGLEGIILKNIDGLWENARSKNLYKFKKVIEVDLKIVGIYPHRKDPTKAGGFILESECGKIKVNAGSGLKDKAGVKSHELDRTRIMENQNYYIGKILECECNGWLKSDGRTDYVKLFLPIAIRLREDKTKANTFEDVFGDFHEVTGL

SEQ ID NO: 22 - protein, 487 aa, Artificial sequence
  Mutant ligase (T4 backbone) protein sequence
MILKILNEIASIGSTKQKQAILEKNKDNELLKRVYRLTYSRGLQYYIKKWPKPGIATQSFGMLTLTDMLDFIEFTLATRKLTGNAAIEELTGYITDGKKDDVEVLRRVMMRDLECGASVSIANKVWPGLIPEQPQMLASSYDEKGINKNIKFPAFAQLKADGARCFAEVRGDELDDVRLLSRAGNEYLGLDLLKEELIKMTAEARQIHPEGVLIDGELVYHEQVKKEPEGLDFLFDAYPENSKAKEFAEVAESRTASNGIANKSLKGTISEKEAQCMKFQVWDYVPLVEIYSLPAFRLKYDVRFSKLEQMTSGYDKVILIENQVVNNLDEAKVIYKKYIDQGLEGIILKNIDGLWENARSKNLYKFKKVIHVDLKIVGIYPHRKDPTKAGGFILESECGKIKVNAGSGLKDKAGVKSHELDRTRIMENQNYYIGKILECECNGWLKSDGRTDYVKLFLPIAIRLREDKTKANTFEDVFGDFHEVTGL

SEQ ID NO: 23 - protein, 482 aa, Artificial sequence
  Mutant ligase (Enterobacteria phage CC31 backbone - clone A4) protein sequence
MILDIINEIASIGSTKEKEAIIRRHKDNELLKRVFRMTYDGKLQYYIKKWDTRPKGDIHLTLEDMLYLLEEKLAKRVVTGNAAKEKLEIALSQTSDADAEVVKKVLLRDLRCGASRSIANKVWKNLIPEQPQMLASSYDEKGIEKNIKFPAFAQLKADGARAFAEVRGDELDDVKILSRAGNEYLGLDLLKQQLIEMTKEARERHPGGVMIDGELVYHASTLPAGPLDDIFGDLPELSKAKEFKEESRTMSNGLANKSLKGTISAKEAAGMKFQVWDYVPLDVVYSEGKQSGFAYDVRFRALELMVQGYSQMILIENHIVHNLDEAKVIYRKYVDEGLEGIILKNIGAFWENTRSKNLYKFKRVIVIDLRIVDIYEHSKQPGKAGGFYLESECGLIKVKAGSGLKDKPGKDAHELDRTRIWENKNDYIGGVLESECNGWLAAEGRTDYVKLFLPIAIKMRRDKDVANTFADIWGDFHEVTGL

SEQ ID NO: 24 - protein, 482 aa, Artificial sequence
  Mutant ligase (Enterobacteria phage CC31 backbone) protein sequence
MILDIINEIASIGSTKEKEAIIRRHKDNELLKRVFRMTYDGKLQYYIKKWDTRPKGDIHLTLEDMLYLLEEKLAKRVVTGNAAKEKLEIALSQTSDADAEVVKKVLLRDLRCGASRSIANKVWKNLIPEQPQMLASSYDEKGIEKNIKFPAFAQLKADGARAFAEVRGDELDDVKILSRAGNEYLGLDLLKQQLIEMTKEARERHPGGVMIDGELVYHASTLPAGPLDDIFGDLPELSKAKEFKEESRTMSNGLANKSLKGTISAKEAAGMKFQVWDYVPLDVVYSEGKQSGFAYDVRFRALELMVQGYSQMILIENHIVHNLDEAKVIYRKYVDEGLEGIILKNIGAFWENTRSKNLYKFKKVIKIDLRIVDIYEHSKQPGKAGGFYLESECGLIKVKAGSGLKDKPGKDAHELDRTRIWENKNDYIGGVLESECNGWLAAEGRTDYVKLFLPIAIKMRRDKDVANTFADIWGDFHEVTGL

SEQ ID NO: 25 - protein, 482 aa, Artificial sequence
  Mutant ligase (Enterobacteria phage CC31 backbone) protein sequence
MILDIINEIASIGSTKEKEAIIRRHKDNELLKRVFRMTYDGKLQYYIKKWDTRPKGDIHLTLEDMLYLLEEKLAKRVVTGNAAKEKLEIALSQTSDADAEVVKKVLLRDLRCGASRSIANKVWKNLIPEQPQMLASSYDEKGIEKNIKFPAFAQLKADGARAFAEVRGDELDDVKILSRAGNEYLGLDLLKQQLIEMTKEARERHPGGVMIDGELVYHASTLPAGPLDDIFGDLPELSKAKEFKEESRTMSNGLANKSLKGTISAKEAAGMKFQVWDYVPLDVVYSEGKQSGFAYDVRFRALELMVQGYSQMILIENHIVHNLDEAKVIYRKYVDEGLEGIILKNIGAFWENTRSKNLYKFKGVIFIDLRIVDIYEHSKQPGKAGGFYLESECGLIKVKAGSGLKDKPGKDAHELDRTRIWENKNDYIGGVLESECNGWLAAEGRTDYVKLFLPIAIKMRRDKDVANTFADIWGDFHEVTGL

SEQ ID NO: 26 - protein, 482 aa, Artificial sequence
  Mutant ligase (Enterobacteria phage CC31 backbone) protein sequence
MILDIINEIASIGSTKEKEAIIRRHKDNELLKRVFRMTYDGKLQYYIKKWDTRPKGDIHLTLEDMLYLLEEKLAKRVVTGNAAKEKLEIALSQTSDADAEVVKKVLLRDLRCGASRSIANKVWKNLIPEQPQMLASSYDEKGIEKNIKFPAFAQLKADGARAFAEVRGDELDDVKILSRAGNEYLGLDLLKQQLIEMTKEARERHPGGVMIDGELVYHASTLPAGPLDDIFGDLPELSKAKEFKEESRTMSNGLANKSLKGTISAKEAAGMKFQVWDYVPLDVVYSEGKQSGFAYDVRFRALELMVQGYSQMILIENHIVHNLDEAKVIYRKYVDEGLEGIILKNIGAFWENTRSKNLYKFKGVILIDLRIVDIYEHSKQPGKAGGFYLESECGLIKVKAGSGLKDKPGKDAHELDRTRIWENKNDYIGGVLESECNGWLAAEGRTDYVKLFLPIAIKMRRDKDVANTFADIWGDFHEVTGL

SEQ ID NO: 27 - protein, 482 aa, Artificial sequence
  Mutant ligase (Enterobacteria phage CC31 backbone) protein sequence
MILDIINEIASIGSTKEKEAIIRRHKDNELLKRVFRMTYDGKLQYYIKKWDTRPKGDIHLTLEDMLYLLEEKLAKRVVTGNAAKEKLEIALSQTSDADAEVVKKVLLRDLRCGASRSIANKVWKNLIPEQPQMLASSYDEKGIEKNIKFPAFAQLKADGARAFAEVRGDELDDVKILSRAGNEYLGLDLLKQQLIEMTKEARERHPGGVMIDGELVYHASTLPAGPLDDIFGDLPELSKAKEFKEESRTMSNGLANKSLKGTISAKEAAGMKFQVWDYVPLDVVYSEGKQSGFAYDVRFRALELMVQGYSQMILIENHIVHNLDEAKVIYRKYVDEGLEGIILKNIGAFWENTRSKNLYKFKRVIFIDLRIVDIYEHSKQPGKAGGFYLESECGLIKVKAGSGLKDKPGKDAHELDRTRIWENKNDYIGGVLESECNGWLAAEGRTDYVKLFLPIAIKMRRDKDVANTFADIWGDFHEVTGL

SEQ ID NO: 28 - protein, 497 aa, Artificial sequence
  Mutant ligase (Shigella phage Shf125875 backbone) protein sequence
MILDILNQIAAIGSTKTKQEILKKNKDNKLLERVYRLTYARGIQYYIKKWPGPGERSQAYGLLELDDMLDFIEFTLATRKLTGNAAIKELMGYIADGKPDDVEVLRRVMMRDLEVGASVSIANKVWPGLIQLQPQMLASAYDEKLITKNIKWPAFAQLKADGARCFAEVRDDGVQFFSRAGNEYHGLTLLADELMEMTKEARERHPNGVLIDGELVYHSFDIKKAVSSGNDLSFLFGDNEESEEVQVADRSTSNGLANKSLQGTISPKEAEGMVLQAWDYVPLDEVYSDGKIKGQKYDVRFAALENMAEGFKRIEPIENQLVHNLDEAKVVYKKYVDQGLEGIILKNRDSYWENKRSKNLIKFKRVIVIALEVVGYYEHSKDPNKLGGVELVSRCRRITTDCGSGFKDTTHKTVDGVKVLIPLDERHDLDRERLMAEAREGKLIGRIADCECNGWVHSKGREGTVGIFLPIIKGFRFDKTEADSFEDVFGPWSQTGL

SEQ ID NO: 29 - protein, 298 aa, Paramecium bursaria Chlorella virus PBCV-1
MAITKPLLAATLENIEDVQFPCLATPKIDGIRSVKQTQMLSRTFKPIRNSVMNRLLTELLPEGSDGEISIEGATFQDTTSAVMTGHKMYNAKFSYYWFDYVTDDPLKKYIDRVEDMKNYITVHPHILEHAQVKIIPLIPVEINNITELLQYERDVLSKGFEGVMIRKPDGKYKFGRSTLKEGILLKMKQFKDAEATIISMTALFKNTNTKTKDNFGYSKRSTHKSGKVEEDVMGSIEVDYDGVVFSIGTGFDADQRRDFWQNKESYIGKMVKFKYFEMGSKDCPRFPVFIGIRHEEDR

SEQ ID NO: 30 - DNA, 23 bp, Artificial sequence
  Example 5, 8 and 9 template oligonucleotide sequence
tttggtgcgaagcagactgaggc

SEQ ID NO: 31 - DNA, 23 bp, Artificial sequence
  Example 5 template oligonucleotide sequence
tttggtgcgaagcagagtgaggc

SEQ ID NO: 32 - DNA, 23 bp, Artificial sequence
  Example 5 template oligonucleotide sequence
tttggtgcgaagcagattgaggc

SEQ ID NO: 33 - DNA, 23 bp, Artificial sequence
  Example 5 template oligonucleotide sequence
tttggtgcgaagcagaatgaggc

SEQ ID NO: 34 - DNA, 23 bp, Artificial sequence
  Example 5 template oligonucleotide sequence
tttggtgcgaagcagtctgaggc

SEQ ID NO: 35 - DNA, 23 bp, Artificial sequence
  Example 5 template oligonucleotide sequence
tttggtgcgaagcagtgtgaggc

SEQ ID NO: 36 - DNA, 23 bp, Artificial sequence
  Example 5 template oligonucleotide sequence
tttggtgcgaagcagtttgaggc

SEQ ID NO: 37 - DNA, 23 bp, Artificial sequence
  Example 5 template oligonucleotide sequence
tttggtgcgaagcagtatgaggc

SEQ ID NO: 38 - DNA, 23 bp, Artificial sequence
  Example 5 template oligonucleotide sequence
tttggtgcgaagcagcctgaggc

SEQ ID NO: 39 - DNA, 23 bp, Artificial sequence
  Example 5 template oligonucleotide sequence
tttggtgcgaagcagcgtgaggc

SEQ ID NO: 40 - DNA, 23 bp, Artificial sequence
  Example 5 template oligonucleotide sequence
tttggtgcgaagcagcttgaggc

SEQ ID NO: 41 - DNA, 23 bp, Artificial sequence
  Example 5 template oligonucleotide sequence
tttggtgcgaagcagcatgaggc

SEQ ID NO: 42 - DNA, 23 bp, Artificial sequence
  Example 5 template oligonucleotide sequence
tttggtgcgaagcaggctgaggc

SEQ ID NO: 43 - DNA, 23 bp, Artificial sequence
  Example 5 template oligonucleotide sequence
tttggtgcgaagcagggtgaggc

SEQ ID NO: 44 - DNA, 23 bp, Artificial sequence
  Example 5 template oligonucleotide sequence
tttggtgcgaagcaggttgaggc

SEQ ID NO: 45 - DNA, 23 bp, Artificial sequence
  Example 5 template oligonucleotide sequence
tttggtgcgaagcaggatgaggc

SEQ ID NO: 46 - DNA, 20 bp, Artificial sequence
  Example 14 "20 mer" oligonucleotide sequence
gccucagtctgcttcgcacc

SEQ ID NO: 47 - DNA, 36 bp, Artificial sequence
  Example 7 template oligonucleotide sequence
tttggtgcgaagcagaaggtaagccgaggtttggcc

SEQ ID NO: 48 - protein, 298 aa, Paramecium bursaria Chlorella virus NE-JV-4
MAITKPLLAATLENIEDVQFPCLATPKIDGIRSVKQTQMLSRTFKPIRNSVMNRLLTELLPEGSDGEISIEGATFQDTTSAVMTGHKMYNAKFSYYWFDYVTDDPLKKYSDRVEDMKNYITAHPHILDHEQVKIIPLIPVEINNITELLQYERDVLSKGFEGVMIRKPDGKYKFGRSTLKEGILLKMKQFKDAEATIISMTALFKNTNTKTKDNFGYSKRSTHKNGKVEEDVMGSIEVDYDGVVFSIGTGFDADQRRDFWQNKESYIGKMVKFKYFEMGSKDCPRFPVFIGIRHEEDH

SEQ ID NO: 49 - protein, 298 aa, Paramecium bursaria Chlorella virus NYs1
MTIAKPLLAATLENLDDVKFPCLVTPKIDGIRSLKQQHMLSRTFKPIRNSVMNKLLSELLPEGADGEICIEDSTFQATTSAVMTGHKVYDEKFSYYWFDYVVDDPLKSYTDRVNDMKKYVDDHPHILEHEQVKIIPLIPVEINNIDELSQYERDVLAKGFEGVMIRRPDGKYKFGRSTLKEGILLKMKQFKDAEATIISMSPRLKNTNAKSKDNLGYSKRSTHKSGKVEEETMGSIEVDYDGVVFSIGTGFDDEQRKHFWENKDSYIGKLLKFKYFEMGSKDAPRFPVFIGIRHEEDC

SEQ ID NO: 50 - protein, 301 aa, Paramecium bursaria Chlorella virus NE-JV-1
MTAIQKPLLAASFKKLTVADVKYPVFATPKLDGIRALKIDGAFVSRTFKPIRNRAIADALQDLLPNGSDGEILSGSTFQDASSAVMTAKAGIGANTIFYWFDYVKDDPNKPYLDRMTDMENYLKERPEILNDDRIKIVPLIPKKIETKDELDTFEKICLDQGFEGVMIRSGAGKYKFGRSTEKEGILIKIKQFEDDEAVVIGFTPMQTNTNDKSMNELGDMKRSSHKDGKVNLDTLGALEVDWNGITFSIGTGFDHALRDKLWSERDKLIGKIVKFKYFAQGVKTAPRFPVFIGFRDPDDM

SEQ ID NO: 51 - protein, 300 aa, Acanthocystis turfacea Chlorella virus Canal-1
MAIQKPLLAASLKKMSVGDLTFPVFATPKLDGIRALKVGGTIVSRTFKPVRNSAISEVLASILPDGSDGEILSGKTFQESTSTVMTADAGLGSGTMFFWFDYVKDDPNKGYLDRIADMKSFTDRHPEILKDKRVTIVPLFPKKIDTTEELHEFEKWCLDQGFEGVMVRNAGGKYKFGRSTEKEQILVKIKQFEDDEAVVIGVSALQTNTNDKKLNQLGEMRRTSHQDGKVELEMLGALDVDWNGIRFSIGTGFDRDTRVDLWKRREGVIGKIVKFKYFSQGIKTAPRFPVFLGFRDKDDM

SEQ ID NO: 52 - protein, 300 aa, Acanthocystis turfacea Chlorella virus Br0604L
MAIQKPLLAASLKKLSVDDLTFPVYATPKLDGIRALKIDGTLVSRTFKPIRNTTISKVLTSLLPDGSDGEILSGKTFQDSTSTVMSADAGIGSGTTFFWFDYVKDDPNKGYLDRIADIKKFIDCRPEILKDSRVIIVPLFPKKIDTAEELNVFEKWCLDQGFEGVMVRNAGGKYKFGRSTEKEQILVKIKQFEDDEAVVIGVSALQTNTNDKKVNELGEMRRTSHQDGKVDLDMLGALDVDWNGIRFGIGTGFDKDTREDLWKRRDSIIGKIVKFKYFSQGVKTAPRFPVFLGFRDKNDM

SEQ ID NO: 53 - protein, 300 aa, Acanthocystis turfacea Chlorella virus NE-JV-2
MAIQKPLLAASLKKLSVDDLTFPVYATPKLDGIRALKIDGTIVSRTFKPIRNTTISNVLMSLLPDGSDGEILSGKTFQDSTSTVMSADAGIGSGTTFFWFDYVKDDPDKGYLDRIADMKKFVDSHPEILKDRRVTIVPLIPKKIDTVEELNVFEQWCLDQGFEGVMVRNAGGKYKFGRSTEKEQILVKIKQFEDDEAVVIGVSALQTNVNDKKMNELGDMRRTSHKDGKIDLEMLGALDVEWNGIRFGIGTGFDKDTREDLWKKRDSIIGKVVKFKYFSQGIKTAPRFPVFLGFRDENDM

SEQ ID NO: 54 - protein, 300 aa, Acanthocystis turfacea Chlorella virus TN603.4.2
MAIQKPLLAASLKKMSVDNLTFPVYATPKLDGIRALKIDGTLVSRTFKPIRNTTISKVLASLLPDGSDGEILSGKTFQDSTSTVMTTDAGIGSDTTFFWFDYVKDDPDKGYLDRIADMKTFVDQHPEILKDSCVTIVPLFPKKIDTPEELHVFEKWCLDQGFEGVMVRTAGGKYKFGRSTEKEQILVKIKQFEDDEAVVIGVSALQTNTNDKKLNQLGEMRRTSHQDGKVDLDMLGALDVDWNGIRFSIGTGFDKDTREDLWKQRDSIVGKVVKFKYFSQGIKTAPRFPVFLGFRDENDM

SEQ ID NO: 55 - protein, 300 aa, Acanthocystis turfacea Chlorella virus GM0701.1
MAIQKPLLAASLKKMSVDDLTFPVYTTPKLDGIRALKIDGTLVSRTFKPVRNSAISEVLASLLPDGSDGEILSGKTFQDSTSTVMTTDAGIGSDTTFFWFDYVKDDPNKGYLDRIADMKTFIDQHPEMLKDNHVTIVPLIPKKIDTVEELNIFEKWCLDQGFEGVMVRNAGGKYKFGRSTEKEQILVKIKQFEDDEAVVIGVSALQTNTNDKKLNQLGEMRRTSHQDGKIDLEMLGALDVDWNGIRFSIGTGFDRDTRVDLWKRRDGIVGRTIKFKYFGQGIKTAPRFPVFLGFRDKDDM

SEQ ID NO: 56 - protein, 287 aa, Synechococcus phage S-CRM01
MLAGNFDPKKAKFPYCATPKIDGIRFLMVNGRALSRTFKPIRNEYIQKLLSKHLPDGIDGELTCGDTFQSSTSAIMRIAGEPDFKAWIFDYVDPDSTSILPFIERFDQISDIIYNGPIPFKHQVLGQSILYNIDDLNRYEEACLNEGYEGVMLRDPYGTYKFGRSSTNEGILLKVKRFEDAEATVIRIDEKMSNQNIAEKDNFGRTKRSSCLDGMVPMETTGALFVRNSDGLEFSIGSGLNDEMRDEIWKNKSSYIGKLVKYKYFPQGVKDLPRHPVFLGFRDPDDM

SEQ ID NO: 57 - protein, 322 aa, marine sediment metagenome
MDAHELMKLNEYAERQNQKQKKQITKPMLAASLKDITQLDYSKGYLATQKLDGIRALMIDGKLVSRTFKPIRNNHIREMLEDVLPDGADGEIVCPGAFQATSSGVMSANGEPEFIYYMFDYVKDDITKEYWRRTQDMVQWLINQGPTRTPGLSKLKLLVPTLIKNYDHLKTYETECIDKGFEGVILRTPDSPYKCGRSTAKQEWLLKLKRFADDEAVVIGFTEKMHNDNEATKDKFGHTVRSSHKENKRPAGTLGSLIVRDIKTEIEFEIGTGFDDELRQKIWDARPEWDGLCVKYKHFAISGVKEKPRFPSFIGVRDVEDM

SEQ ID NO: 58 - protein, 691 aa, Mycobacterium tuberculosis (strain ATCC 25618/H37Rv)
MSSPDADQTAPEVLRQWQALAEEVREHQFRYYVRDAPIISDAEFDELLRRLEALEEQHPELRTPDSPTQLVGGAGFATDFEPVDHLERMLSLDNAFTADELAAWAGRIHAEVGDAAHYLCELKIDGVALSLVYREGRLTRASTRGDGRTGEDVTLNARTIADVPERLTPGDDYPVPEVLEVRGEVFFRLDDFQALNASLVEEGKAPFANPRNSAAGSLRQKDPAVTARRRLRMICHGLGHVEGFRPATLHQAYLALRAWGLPVSEHTTLATDLAGVRERIDYWGEHRHEVDHEIDGVVVKVDEVALQRRLGSTSRAPRWAIAYKYPPEEAQTKLLDIRVNVGRTGRITPFAFMTPVKVAGSTVGQATLHNASEIKRKGVLIGDTVVIRKAGDVIPEVLGPVVELRDGSEREFIMPTTCPECGSPLAPEKEGDADIRCPNARGCPGQLRERVFHVASRNGLDIEVLGYEAGVALLQAKVIADEGELFALTERDLLRTDLFRTKAGELSANGKRLLVNLDKAKAAPLWRVLVALSIRHVGPTAARALATEFGSLDAIAAASTDQLAAVEGVGPTIAAAVTEWFAVDWHREIVDKWRAAGVRMVDERDESVPRTLAGLTIVVTGSLTGFSRDDAKEAIVARGGKAAGSVSKKTNYVVAGDSPGSKYDKAVELGVPILDEDGFRRLLADGPASRT

SEQ ID NO: 59 - protein, 676 aa, Enterococcus faecalis (strain ATCC 700802/V583)
MEQQPLTLTAATTRAQELRKQLNQYSHEYYVKDQPSVEDYVYDRLYKELVDIETEFPDLITPDSPTQRVGGKVLSGFEKAPHDIPMYSLNDGFSKEDIFAFDERVRKAIGKPVAYCCELKIDGLAISLRYENGVFVRGATRGDGTVGENITENLRTVRSVPMRLTEPISVEVRGECYMPKQSFVALNEEREENGQDIFANPRNAAAGSLRQLDTKIVAKRNLNTFLYTVADFGPMKAKTQFEALEELSAIGFRTNPERQLCQSIDEVWAYIEEYHEKRSTLPYEIDGIVIKVNEFALQDELGFTVKAPRWAIAYKFPPEEAETVVEDIEWTIGRTGVVTPTAVMAPVRVAGTTVSRASLHNADFIQMKDIRLNDHVIIYKAGDIIPEVAQVLVEKRAADSQPYEMPTHCPICHSELVHLDEEVALRCINPKCPAQIKEGLNHFVSRNAMNIDGLGPRVLAQMYDKGLVKDVADLYFLTEEQLMTLDKIKEKSANNIYTAIQGSKENSVERLIFGLGIRHVGAKAAKILAEHFGDLPTLSRATAEEIVALDSIGETIADSVVTYFENEEVHELMAELEKAQVNLTYKGLRTEQLAEVESPFKDKTVVLTGKLAQYTREEAKEKIENLGGKVTGSVSKKTDIVVAGEDAGSKLTKAESLGVTVWNEQEMVDALDASHF

SEQ ID NO: 60 - protein, 670 aa, Haemophilus influenzae (strain ATCC 51907/DSM 11121/ KW20/Rd)
MTNIQTQLDNLRKTLRQYEYEYHVLDNPSVPDSEYDRLFHQLKALELEHPEFLTSDSPTQRVGAKPLSGFSQIRHEIPMLSLDNAFSDAEFNAFVKRIEDRLILLPKPLTFCCEPKLDGLAVSILYVNGELTQAATRGDGTTGEDITANIRTIRNVPLQLLTDNPPARLEVRGEVFMPHAGFERLNKYALEHNEKTFANPRNAAAGSLRQLDPNITSKRPLVLNAYGIGIAEGVDLPTTHYARLQWLKSIGIPVNPEIRLCNGADEVLGFYRDIQNKRSSLGYDIDGTVLKINDIALQNELGFISKAPRWAIAYKFPAQEELTLLNDVEFQVGRTGAITPVAKLEPVFVAGVTVSNATLHNGDEIERLNIAIGDTVVIRRAGDVIPQIIGVLHERRPDNAKPIIFPTNCPVCDSQIIRIEGEAVARCTGGLFCAAQRKEALKHFVSRKAMDIDGVGGKLIEQLVDRELIHTPADLFKLDLTTLTRLERMGAKSAENALNSLENAKSTTLARFIFALGIREVGEATALNLANHFKTLDALKDANLEELQQVPDVGEVVANRIFIFWREAHNVAVVEDLIAQGVHWETVEVKEASENLFKDKTVVLTGTLTQMGRNEAKALLQQLGAKVSGSVSSKTDFVIAGDAAGSKLAKAQELNITVLTEEEFLAQITR

SEQ ID NO: 61 - protein, 667 aa, Staphylococcus aureus
MADLSSRVNELHDLLNQYSYEYYVEDNPSVPDSEYDKLLHELIKIEEEHPEYKTVDSPTVRVGGEAQASFNKVNHDTPMLSLGNAFNEDDLRKFDQRIREQIGNVEYMCELKIDGLAVSLKYVDGYFVQGLTRGDGTTGEDITENLKTIHAIPLKMKEPLNVEVRGEAYMPRRSFLRLNEEKEKNDEQLFANPRNAAAGSLRQLDSKLTAKRKLSVFIYSVNDFTDFNARSQSEALDELDKLGFTTNKNRARVNNIDGVLEYIEKWTSQRESLPYDIDGIVIKVNDLDQQDEMGFTQKSPRWAIAYKFPAEEVVTKLLDIELSIGRTGVVTPTAILEPVKVAGTTVSRASLHNEDLIHDRDIRIGDSVVVKKAGDIIPEVVRSIPERRPEDAVTYHMPTHCPSCGHELVRIEGEVALRCINPKCQAQLVEGLIHFVSRQAMNIDGLGTKIIQQLYQSELIKDVADIFYLTEEDLLPLDRMGQKKVDNLLAAIQQAKDNSLENLLFGLGIRHLGVKASQVLAEKYETIDRLLTVTEAELVEIHDIGDKVAQSVVTYLENEDIRALIQKLKDKHVNMIYKGIKTSDIEGHPEFSGKTIVLTGKLHQMTRNEASKWLASQGAKVTSSVTKNTDVVIAGEDAGSKLTKAQSLGIEIWTEQQFVDKQNELNS

SEQ ID NO: 62 - protein, 652 aa, Streptococcus pneumoniae (strain P1031)
MNKRMNELVALLNRYATEYYTSDNPSVSDSEYDRLYRELVELETAYPEQVLADSPTHRVGGKVLDGFEKYSHQYPLYSLQDAFSREELDAFDARVRKEVAHPTYICELKIDGLSISLTYEKGILVAGVTRGDGSIGENITENLKRVKDIPLTLPEELDITVRGECYMPRASFDQVNQARQENGEPEFANPRNAAAGTLRQLDTAVVAKRNLATFLYQEASPSTRDSQEKGLKYLEQLGFVVNPKRILAENIDEIWNFIQEVGQERENLPYDIDGVVIKVNDLASQEELGFTVKAPKWAVAYKFPAEEKEAQLLSVDWTVGRTGVVTPTANLTPVQLAGTTVSRATLHNVDYIAEKDIRKDDTVIVYKAGDIIPAVLRVVESKRVSEEKLDIPTNCPSCNSDLLHFEDEVALRCINPRCPAQIMEGLIHFASRDAMNITGLGPSIVEKLFAANLVKDVADIYRLQEEDFLLLEGVKEKSAAKLYQAIQASKENSAEKLLFGLGIRHVGSKASQLLLQYFHSIENLYQADSEEVASIESLGGVIAKSLQTYFATEGSEILLRELKETGVNLDYKGQTVVADAALSGLTVVLTGKLERLKRSEAKSKLESLGAKVTGSVSKKTDLVVVGADAGSKLQKAQELGIQVRDEAWLESL